European Patent Application EP 4 116 415 A1, published January 11, 2023. Title: NEURODEGENERATIVE DISORDERS. Applicant: Neuro-Bio Ltd. The sequence listing filed with the application follows.

SEQUENCE LISTING (158 sequences)

SEQ ID NO: 1 - protein, 14 aa, Homo sapiens
AEFHRWSSYMVHWK

SEQ ID NO: 2 - protein, 4 aa, Artificial Sequence
  A peptide according to the invention
HWKA

SEQ ID NO: 3 - protein, 4 aa, Artificial Sequence
  A peptide according to the invention
WKAE

SEQ ID NO: 4 - protein, 4 aa, Artificial Sequence
  A peptide according to the invention
KAEF

SEQ ID NO: 5 - protein, 4 aa, Artificial Sequence
  A peptide according to the invention
AEFH

SEQ ID NO: 6 - protein, 4 aa, Artificial Sequence
  A peptide according to the invention
EFHR

SEQ ID NO: 7 - protein, 4 aa, Artificial Sequence
  A peptide according to the invention
FHRW

SEQ ID NO: 8 - protein, 4 aa, Artificial Sequence
  A peptide according to the invention
HRWS

SEQ ID NO: 9 - protein, 4 aa, Artificial Sequence
  A peptide according to the invention
RWSS

SEQ ID NO: 10 - protein, 4 aa, Artificial Sequence
  A peptide according to the invention
WSSY

SEQ ID NO: 11 - protein, 4 aa, Artificial Sequence
  A peptide according to the invention
SSYM

SEQ ID NO: 12 - protein, 4 aa, Artificial Sequence
  A peptide according to the invention
SYMV

SEQ ID NO: 13 - protein, 4 aa, Artificial Sequence
  A peptide according to the invention
YMVH

SEQ ID NO: 14 - protein, 4 aa, Artificial Sequence
  A peptide according to the invention
MVHW

SEQ ID NO: 15 - protein, 4 aa, Artificial Sequence
  A peptide according to the invention
VHWK

SEQ ID NO: 16 - protein, 5 aa, Artificial Sequence
  A peptide according to the invention
HWKAE

SEQ ID NO: 17 - protein, 5 aa, Artificial Sequence
  A peptide according to the invention
WKAEF

SEQ ID NO: 18 - protein, 5 aa, Artificial Sequence
  A peptide according to the invention
KAEFH

SEQ ID NO: 19 - protein, 5 aa, Artificial Sequence
  A peptide according to the invention
AEFHR

SEQ ID NO: 20 - protein, 5 aa, Artificial Sequence
  A peptide according to the invention
EFHRW

SEQ ID NO: 21 - protein, 5 aa, Artificial Sequence
  A peptide according to the invention
FHRWS

SEQ ID NO: 22 - protein, 5 aa, Artificial Sequence
  A peptide according to the invention
HRWSS

SEQ ID NO: 23 - protein, 5 aa, Artificial Sequence
  A peptide according to the invention
RWSSY

SEQ ID NO: 24 - protein, 5 aa, Artificial Sequence
  A peptide according to the invention
WSSYM

SEQ ID NO: 25 - protein, 5 aa, Artificial Sequence
  A peptide according to the invention
SSYMV

SEQ ID NO: 26 - protein, 5 aa, Artificial Sequence
  A peptide according to the invention
SYMVH

SEQ ID NO: 27 - protein, 5 aa, Artificial Sequence
  A peptide according to the invention
YMVHW

SEQ ID NO: 28 - protein, 5 aa, Artificial Sequence
  A peptide according to the invention
MVHWK

SEQ ID NO: 29 - protein, 5 aa, Artificial Sequence
  A peptide according to the invention
VHWKA

SEQ ID NO: 30 - protein, 6 aa, Artificial Sequence
  A peptide according to the invention
HWKAEF

SEQ ID NO: 31 - protein, 6 aa, Artificial Sequence
  A peptide according to the invention
WKAEFH

SEQ ID NO: 32 - protein, 6 aa, Artificial Sequence
  A peptide according to the invention
KAEFHR

SEQ ID NO: 33 - protein, 6 aa, Artificial Sequence
  A peptide according to the invention
AEFHRW

SEQ ID NO: 34 - protein, 6 aa, Artificial Sequence
  A peptide according to the invention
EFHRWS

SEQ ID NO: 35 - protein, 6 aa, Artificial Sequence
  A peptide according to the invention
FHRWSS

SEQ ID NO: 36 - protein, 6 aa, Artificial Sequence
  A peptide according to the invention
HRWSSY

SEQ ID NO: 37 - protein, 6 aa, Artificial Sequence
  A peptide according to the invention
RWSSYM

SEQ ID NO: 38 - protein, 6 aa, Artificial Sequence
  A peptide according to the invention
WSSYMV

SEQ ID NO: 39 - protein, 6 aa, Artificial Sequence
  A peptide according to the invention
SSYMVH

SEQ ID NO: 40 - protein, 6 aa, Artificial Sequence
  A peptide according to the invention
SYMVHW

SEQ ID NO: 41 - protein, 6 aa, Artificial Sequence
  A peptide according to the invention
YMVHWK

SEQ ID NO: 42 - protein, 6 aa, Artificial Sequence
  A peptide according to the invention
MVHWKA

SEQ ID NO: 43 - protein, 6 aa, Artificial Sequence
  A peptide according to the invention
VHWKAE

SEQ ID NO: 44 - protein, 7 aa, Artificial Sequence
  A peptide according to the invention
HWKAEFH

SEQ ID NO: 45 - protein, 7 aa, Artificial Sequence
  A peptide according to the invention
WKAEFHR

SEQ ID NO: 46 - protein, 7 aa, Artificial Sequence
  A peptide according to the invention
KAEFHRW

SEQ ID NO: 47 - protein, 7 aa, Artificial Sequence
  A peptide according to the invention
AEFHRWS

SEQ ID NO: 48 - protein, 7 aa, Artificial Sequence
  A peptide according to the invention
EFHRWSS

SEQ ID NO: 49 - protein, 7 aa, Artificial Sequence
  A peptide according to the invention
FHRWSSY

SEQ ID NO: 50 - protein, 7 aa, Artificial Sequence
  A peptide according to the invention
HRWSSYM

SEQ ID NO: 51 - protein, 7 aa, Artificial Sequence
  A peptide according to the invention
RWSSYMV

SEQ ID NO: 52 - protein, 7 aa, Artificial Sequence
  A peptide according to the invention
WSSYMVH

SEQ ID NO: 53 - protein, 7 aa, Artificial Sequence
  A peptide according to the invention
SSYMVHW

SEQ ID NO: 54 - protein, 7 aa, Artificial Sequence
  A peptide according to the invention
SYMVHWK

SEQ ID NO: 55 - protein, 7 aa, Artificial Sequence
  A peptide according to the invention
YMVHWKA

SEQ ID NO: 56 - protein, 7 aa, Artificial Sequence
  A peptide according to the invention
MVHWKAE

SEQ ID NO: 57 - protein, 7 aa, Artificial Sequence
  A peptide according to the invention
VHWKAEF

SEQ ID NO: 58 - protein, 8 aa, Artificial Sequence
  A peptide according to the invention
HWKAEFHR

SEQ ID NO: 59 - protein, 8 aa, Artificial Sequence
  A peptide according to the invention
WKAEFHRW

SEQ ID NO: 60 - protein, 8 aa, Artificial Sequence
  A peptide according to the invention
KAEFHRWS

SEQ ID NO: 61 - protein, 8 aa, Artificial Sequence
  A peptide according to the invention
AEFHRWSS

SEQ ID NO: 62 - protein, 8 aa, Artificial Sequence
  A peptide according to the invention
EFHRWSSY

SEQ ID NO: 63 - protein, 8 aa, Artificial Sequence
  A peptide according to the invention
FHRWSSYM

SEQ ID NO: 64 - protein, 8 aa, Artificial Sequence
  A peptide according to the invention
HRWSSYMV

SEQ ID NO: 65 - protein, 8 aa, Artificial Sequence
  A peptide according to the invention
RWSSYMVH

SEQ ID NO: 66 - protein, 8 aa, Artificial Sequence
  A peptide according to the invention
WSSYMVHW

SEQ ID NO: 67 - protein, 8 aa, Artificial Sequence
  A peptide according to the invention
SSYMVHWK

SEQ ID NO: 68 - protein, 8 aa, Artificial Sequence
  A peptide according to the invention
SYMVHWKA

SEQ ID NO: 69 - protein, 8 aa, Artificial Sequence
  A peptide according to the invention
YMVHWKAE

SEQ ID NO: 70 - protein, 8 aa, Artificial Sequence
  A peptide according to the invention
MVHWKAEF

SEQ ID NO: 71 - protein, 8 aa, Artificial Sequence
  A peptide according to the invention
VHWKAEFH

SEQ ID NO: 72 - protein, 9 aa, Artificial Sequence
  A peptide according to the invention
HWKAEFHRW

SEQ ID NO: 73 - protein, 9 aa, Artificial Sequence
  A peptide according to the invention
WKAEFHRWS

SEQ ID NO: 74 - protein, 9 aa, Artificial Sequence
  A peptide according to the invention
KAEFHRWSS

SEQ ID NO: 75 - protein, 9 aa, Artificial Sequence
  A peptide according to the invention
AEFHRWSSY

SEQ ID NO: 76 - protein, 9 aa, Artificial Sequence
  A peptide according to the invention
EFHRWSSYM

SEQ ID NO: 77 - protein, 9 aa, Artificial Sequence
  A peptide according to the invention
FHRWSSYMV

SEQ ID NO: 78 - protein, 9 aa, Artificial Sequence
  A peptide according to the invention
HRWSSYMVH

SEQ ID NO: 79 - protein, 9 aa, Artificial Sequence
  A peptide according to the invention
RWSSYMVHW

SEQ ID NO: 80 - protein, 9 aa, Artificial Sequence
  A peptide according to the invention
WSSYMVHWK

SEQ ID NO: 81 - protein, 9 aa, Artificial Sequence
  A peptide according to the invention
SSYMVHWKA

SEQ ID NO: 82 - protein, 9 aa, Artificial Sequence
  A peptide according to the invention
SYMVHWKAE

SEQ ID NO: 83 - protein, 9 aa, Artificial Sequence
  A peptide according to the invention
YMVHWKAEF

SEQ ID NO: 84 - protein, 9 aa, Artificial Sequence
  A peptide according to the invention
MVHWKAEFH

SEQ ID NO: 85 - protein, 9 aa, Artificial Sequence
  A peptide according to the invention
VHWKAEFHR

SEQ ID NO: 86 - protein, 10 aa, Artificial Sequence
  A peptide according to the invention
HWKAEFHRWS

SEQ ID NO: 87 - protein, 10 aa, Artificial Sequence
  A peptide according to the invention
WKAEFHRWSS

SEQ ID NO: 88 - protein, 10 aa, Artificial Sequence
  A peptide according to the invention
KAEFHRWSSY

SEQ ID NO: 89 - protein, 10 aa, Artificial Sequence
  A peptide according to the invention
AEFHRWSSYM

SEQ ID NO: 90 - protein, 10 aa, Artificial Sequence
  A peptide according to the invention
EFHRWSSYMV

SEQ ID NO: 91 - protein, 10 aa, Artificial Sequence
  A peptide according to the invention
FHRWSSYMVH

SEQ ID NO: 92 - protein, 10 aa, Artificial Sequence
  A peptide according to the invention
HRWSSYMVHW

SEQ ID NO: 93 - protein, 10 aa, Artificial Sequence
  A peptide according to the invention
HRWSSYMVHW

SEQ ID NO: 94 - protein, 10 aa, Artificial Sequence
  A peptide according to the invention
WSSYMVHWKA

SEQ ID NO: 95 - protein, 10 aa, Artificial Sequence
  A peptide according to the invention
SSYMVHWKAE

SEQ ID NO: 96 - protein, 10 aa, Artificial Sequence
  A peptide according to the invention
SYMVHWKAEF

SEQ ID NO: 97 - protein, 10 aa, Artificial Sequence
  A peptide according to the invention
YMVHWKAEFH

SEQ ID NO: 98 - protein, 10 aa, Artificial Sequence
  A peptide according to the invention
MVHWKAEFHR

SEQ ID NO: 99 - protein, 10 aa, Artificial Sequence
  A peptide according to the invention
VHWKAEFHRW

SEQ ID NO: 100 - protein, 11 aa, Artificial Sequence
  A peptide according to the invention
HWKAEFHRWSS

SEQ ID NO: 101 - protein, 11 aa, Artificial Sequence
  A peptide according to the invention
WKAEFHRWSSY

SEQ ID NO: 102 - protein, 11 aa, Artificial Sequence
  A peptide according to the invention
KAEFHRWSSYM

SEQ ID NO: 103 - protein, 11 aa, Artificial Sequence
  A peptide according to the invention
AEFHRWSSYMV

SEQ ID NO: 104 - protein, 11 aa, Artificial Sequence
  A peptide according to the invention
EFHRWSSYMVH

SEQ ID NO: 105 - protein, 11 aa, Artificial Sequence
  A peptide according to the invention
FHRWSSYMVHW

SEQ ID NO: 106 - protein, 11 aa, Artificial Sequence
  A peptide according to the invention
HRWSSYMVHWK

SEQ ID NO: 107 - protein, 11 aa, Artificial Sequence
  A peptide according to the invention
RWSSYMVHWKA

SEQ ID NO: 108 - protein, 11 aa, Artificial Sequence
  A peptide according to the invention
WSSYMVHWKAE

SEQ ID NO: 109 - protein, 11 aa, Artificial Sequence
  A peptide according to the invention
SSYMVHWKAEF

SEQ ID NO: 110 - protein, 11 aa, Artificial Sequence
  A peptide according to the invention
SYMVHWKAEFH

SEQ ID NO: 111 - protein, 11 aa, Artificial Sequence
  A peptide according to the invention
YMVHWKAEFHR

SEQ ID NO: 112 - protein, 11 aa, Artificial Sequence
  A peptide according to the invention
MVHWKAEFHRW

SEQ ID NO: 113 - protein, 11 aa, Artificial Sequence
  A peptide according to the invention
VHWKAEFHRWS

SEQ ID NO: 114 - protein, 12 aa, Artificial Sequence
  A peptide according to the invention
HWKAEFHRWSSY

SEQ ID NO: 115 - protein, 12 aa, Artificial Sequence
  A peptide according to the invention
WKAEFHRWSSYM

SEQ ID NO: 116 - protein, 12 aa, Artificial Sequence
  A peptide according to the invention
KAEFHRWSSYMV

SEQ ID NO: 117 - protein, 12 aa, Artificial Sequence
  A peptide according to the invention
AEFHRWSSYMVH

SEQ ID NO: 118 - protein, 12 aa, Artificial Sequence
  A peptide according to the invention
EFHRWSSYMVHW

SEQ ID NO: 119 - protein, 12 aa, Artificial Sequence
  A peptide according to the invention
FHRWSSYMVHWK

SEQ ID NO: 120 - protein, 12 aa, Artificial Sequence
  A peptide according to the invention
HRWSSYMVHWKA

SEQ ID NO: 121 - protein, 12 aa, Artificial Sequence
  A peptide according to the invention
RWSSYMVHWKAE

SEQ ID NO: 122 - protein, 12 aa, Artificial Sequence
  A peptide according to the invention
WSSYMVHWKAEF

SEQ ID NO: 123 - protein, 12 aa, Artificial Sequence
  A peptide according to the invention
SSYMVHWKAEFH

SEQ ID NO: 124 - protein, 12 aa, Artificial Sequence
  A peptide according to the invention
SYMVHWKAEFHR

SEQ ID NO: 125 - protein, 12 aa, Artificial Sequence
  A peptide according to the invention
YMVHWKAEFHRW

SEQ ID NO: 126 - protein, 12 aa, Artificial Sequence
  A peptide according to the invention
MVHWKAEFHRWS

SEQ ID NO: 127 - protein, 12 aa, Artificial Sequence
  A peptide according to the invention
VHWKAEFHRWSS

SEQ ID NO: 128 - protein, 13 aa, Artificial Sequence
  A peptide according to the invention
HWKAEFHRWSSYM

SEQ ID NO: 129 - protein, 13 aa, Artificial Sequence
  A peptide according to the invention
WKAEFHRWSSYMV

SEQ ID NO: 130 - protein, 13 aa, Artificial Sequence
  A peptide according to the invention
KAEFHRWSSYMVH

SEQ ID NO: 131 - protein, 13 aa, Artificial Sequence
  A peptide according to the invention
AEFHRWSSYMVHW

SEQ ID NO: 132 - protein, 13 aa, Artificial Sequence
  A peptide according to the invention
EFHRWSSYMVHWK

SEQ ID NO: 133 - protein, 13 aa, Artificial Sequence
  A peptide according to the invention
FHRWSSYMVHWKA

SEQ ID NO: 134 - protein, 13 aa, Artificial Sequence
  A peptide according to the invention
HRWSSYMVHWKAE

SEQ ID NO: 135 - protein, 13 aa, Artificial Sequence
  A peptide according to the invention
RWSSYMVHWKAEF

SEQ ID NO: 136 - protein, 13 aa, Artificial Sequence
  A peptide according to the invention
WSSYMVHWKAEFH

SEQ ID NO: 137 - protein, 13 aa, Artificial Sequence
  A peptide according to the invention
SSYMVHWKAEFHR

SEQ ID NO: 138 - protein, 13 aa, Artificial Sequence
  A peptide according to the invention
SYMVHWKAEFHRW

SEQ ID NO: 139 - protein, 13 aa, Artificial Sequence
  A peptide according to the invention
YMVHWKAEFHRWS

SEQ ID NO: 140 - protein, 13 aa, Artificial Sequence
  A peptide according to the invention
MVHWKAEFHRWSS

SEQ ID NO: 141 - protein, 13 aa, Artificial Sequence
  A peptide according to the invention
VHWKAEFHRWSSY

SEQ ID NO: 142 - protein, 14 aa, Artificial Sequence
  A peptide according to the invention
HWKAEFHRWSSYMV

SEQ ID NO: 143 - protein, 14 aa, Artificial Sequence
  A peptide according to the invention
WKAEFHRWSSYMVH

SEQ ID NO: 144 - protein, 14 aa, Artificial Sequence
  A peptide according to the invention
KAEFHRWSSYMVHW

SEQ ID NO: 145 - protein, 14 aa, Artificial Sequence
  A peptide according to the invention
AEFHRWSSYMVHWK

SEQ ID NO: 146 - protein, 14 aa, Artificial Sequence
  A peptide according to the invention
EFHRWSSYMVHWKA

SEQ ID NO: 147 - protein, 14 aa, Artificial Sequence
  A peptide according to the invention
FHRWSSYMVHWKAE

SEQ ID NO: 148 - protein, 14 aa, Artificial Sequence
  A peptide according to the invention
HRWSSYMVHWKAEF

SEQ ID NO: 149 - protein, 14 aa, Artificial Sequence
  A peptide according to the invention
RWSSYMVHWKAEFH

SEQ ID NO: 150 - protein, 14 aa, Artificial Sequence
  A peptide according to the invention
WSSYMVHWKAEFHR

SEQ ID NO: 151 - protein, 14 aa, Artificial Sequence
  A peptide according to the invention
SSYMVHWKAEFHRW

SEQ ID NO: 152 - protein, 14 aa, Artificial Sequence
  A peptide according to the invention
SYMVHWKAEFHRWS

SEQ ID NO: 153 - protein, 14 aa, Artificial Sequence
  A peptide according to the invention
YMVHWKAEFHRWSS

SEQ ID NO: 154 - protein, 14 aa, Artificial Sequence
  A peptide according to the invention
MVHWKAEFHRWSSY

SEQ ID NO: 155 - protein, 14 aa, Artificial Sequence
  A peptide according to the invention
VHWKAEFHRWSSYM

SEQ ID NO: 156 - protein, 30 aa, Artificial Sequence
  Linear, T30 peptide
KAEFHRWSSYMVHWKNQFDHYSKQDRCSDL

SEQ ID NO: 157 - protein, 614 aa, Artificial Sequence
  Amino acid sequence of the tail of human acetylcholinesterase
MRPPQCLLHTPSLASPLLLLLLWLLGGGVGAEGREDAELLVTVRGGRLRGIRLKTPGGPVSAFLGIPFAEPPMGPRRFLPPEPKQPWSGVVDATTFQSVCYQYVDTLYPGFEGTEMWNPNRELSEDCLYLNVWTPYPRPTSPTPVLVWIYGGGFYSGASSLDVYDGRFLVQAERTVLVSMNYRVGAFGFLALPGSREAPGNVGLLDQRLALQWVQENVAAFGGDPTSVTLFGESAGAASVGMHLLSPPSRGLFHRAVLQSGAPNGPWATVGMGEARRRATQLAHLVGCPPGGTGGNDTELVACLRTRPAQVLVNHEWHVLPQESVFRFSFVPVVDGDFLSDTPEALINAGDFHGLQVLVGVVKDEGSYFLVYGAPGFSKDNESLISRAEFLAGVRVGVPQVSDLAAEAVVLHYTDWLHPEDPARLREALSDVVGDHNVVCPVAQLAGRLAAQGARVYAYVFEHRASTLSWPLWMGVPHGYEIEFIFGIPLDPSRNYTAEEKIFAQRLMRYWANFARTGDPNEPRDPKAPQWPPYTAGAQQYVSLDLRPLEVRRGLRAQACAFWNRFLPKLLSATDTLDEAERQWKAEFHRWSSYMVHWKNQFDHYSKQDRCSDL

SEQ ID NO: 158 - protein, 42 aa, Artificial Sequence [sequence omitted]